European Patent Specification EP 3 917 881 B9, published September 27, 2023. Title: Maskierung von kristallinem Siliciumdioxid. Applicant: Quarzwerke. The sequence listing filed with the application follows.

SEQUENCE LISTING (2 sequences)

SEQ ID NO: 1 - DNA, 20 bp, Artificial Sequence
  Primer
ctgtcatgtcgaccctcagt

SEQ ID NO: 2 - DNA, 20 bp, Artificial Sequence
  Primer
tcgagcaagtctttcagtcc